European Patent Application EP 4 174 166 A1, published May 3, 2023. Title: Novel Faecalibacterium prausnitzii EB-FPDK9 and Use Thereof. Applicant: Enterobiome Co., Ltd. The sequence listing filed with the application follows.

SEQUENCE LISTING (26 sequences)

SEQ ID NO: 1 - DNA, 1433 bp, Artificial Sequence
  Faecalibacterium prausnitzii EB-RPDK9 16S rRNA
gacgaacgctggcggcgcgcctaacacatgcaagtcgaacgagcgagagagagcttgctttctcgagcgagtggcgaacgggtgagtaacgcgtgaggaacctgcctcaaagagggggacaacagttggaaacgactgctaataccgcataagcccacgactcggcatcgggtagagggaaaaggagcaatccgctttgagatggcctcgcgtccgattagctagttggtgaggtaacggcccaccaaggcgacgatcggtagccggactgagaggttgaacggccacattgggactgagacacggcccagactcctacgggaggcagcagtggggaatattgcacaatgggggaaaccctgatgcagcgacgccgcgtggaggaagaaggtcttcggattgtaaactcctgttgttgaggaagataatgacggtactcaacaaggaagtgacggctaactacgtgccagcagccgcggtaaaacgtaggtcacaagcgttgtccggaattactgggtgtaaagggagcgcaggcgggaagacaagttggaagtgaaatccatgggctcaacccatgaactgctttcaaaactgtttttcttgagtagtgcagaggtaggcggaattcccggtgtagcggtggaatgcgtagatatcgggaggaacaccagtggcgaaggcggcctactgggcaccaactgacgctgaggctcgaaagtgtgggtagcaaacaggattagataccctggtagtccacactgtaaacgatgattactaggtgttggaggattgaccccttcagtgccgcagttaacacaataagtaatccacctggggagtacgaccgcaaggttgaaactcaaaggaattgacgggggcccgcacaagcagtggagtatgtggtttaattcgacgcaacgcgaagaaccttaccaagtcttgacatcctgcgacgcacatagaaatatgtgtttccttcgggacgcagagacaggtggtgcatggttgtcgtcagctcgtgtcgtgagatgttgggttaagtcccgcaacgagcgcaacccttatggtcagttactacgcaagaggactctggccagactgccgttgacaaaacggaggaaggtggggatgacgtcaaatcatcatgccctttatgacttgggctacacacgtactacaatggcgttaaacaaagagaagcaagaccgcgaggtggagcaaaactcagaaacaacgtcccagttcggactgcaggctgcaactcgcctgcacgaagtcggaattgctagtaatcgcagatcagcatgctgcggtgaatacgttcccgggccttgtacacaccgcccgtcacaccatgagagccggggggacccgaagtcggtagtctaaccgcaaggaggacgccgccgaaggtaaaactggtgattggggtg

SEQ ID NO: 2 - DNA, 17 bp, Artificial Sequence
  FP1 Forward
actcaacaaggaagtga

SEQ ID NO: 3 - DNA, 17 bp, Artificial Sequence
  FP2 Reverse
cagaggtaggcggaatt

SEQ ID NO: 4 - DNA, 22 bp, Artificial Sequence
  ERIC-1 Forward
atgtaagctcctggggattcac

SEQ ID NO: 5 - DNA, 22 bp, Artificial Sequence
  ERIC-2 Reverse
aagtaagtgactggggtgagcg

SEQ ID NO: 6 - DNA, 15 bp, Artificial Sequence
  (GTG)5 Forward/Reverse
gtggtggtggtggtg

SEQ ID NO: 7 - DNA, 20 bp, Artificial Sequence
  27F Forward
agagtttgatcmtggctcag

SEQ ID NO: 8 - DNA, 19 bp, Artificial Sequence
  1492R Reverse
ggttaccttgttacgactt

SEQ ID NO: 9 - DNA, 24 bp, Artificial Sequence
  GAPDH Forward
gacatcaagaaggtggtgaagcag

SEQ ID NO: 10 - DNA, 24 bp, Artificial Sequence
  GAPDH Reverse
ataccaggaaatgagcttgacaaa

SEQ ID NO: 11 - DNA, 22 bp, Artificial Sequence
  IL-8 Forward
ttttgccaaggagtgctaaaga

SEQ ID NO: 12 - DNA, 21 bp, Artificial Sequence
  IL-8 Reverse
aaccctctgcacccagttttc

SEQ ID NO: 13 - DNA, 24 bp, Artificial Sequence
  GAPDH Forward
gacatcaagaaggtggtgaagcag

SEQ ID NO: 14 - DNA, 24 bp, Artificial Sequence
  GAPDH Reverse
ataccaggaaatgagcttgacaaa

SEQ ID NO: 15 - DNA, 20 bp, Artificial Sequence
  C/EBPa Forward
agcaacgagtaccgggtacg

SEQ ID NO: 16 - DNA, 21 bp, Artificial Sequence
  C/EBPa Reverse
tgtttggctttatctcggctc

SEQ ID NO: 17 - DNA, 17 bp, Artificial Sequence
  SREBP1c Forward
gatgtgcgaactggaca

SEQ ID NO: 18 - DNA, 19 bp, Artificial Sequence
  SREBP1c Reverse
catagggggcgtcaaacag

SEQ ID NO: 19 - DNA, 26 bp, Artificial Sequence
  aP2 Forward
agtgaaaacttcgatgattacatgaa

SEQ ID NO: 20 - DNA, 19 bp, Artificial Sequence
  aP2 Reverse
gcctgccactttccttgtg

SEQ ID NO: 21 - DNA, 20 bp, Artificial Sequence
  FAS Foward
aggggtcgacctggtcctca

SEQ ID NO: 22 - DNA, 20 bp, Artificial Sequence
  FAS Reverse
gccatgcccagagggtggtt

SEQ ID NO: 23 - DNA, 20 bp, Artificial Sequence
  ACC1 Forward
cctccgtcagctcagataca

SEQ ID NO: 24 - DNA, 22 bp, Artificial Sequence
  ACC1 Reverse
tttactaggtgcaagccagaca

SEQ ID NO: 25 - DNA, 20 bp, Artificial Sequence
  LPL Forward
ttgccctaaggacccctgaa

SEQ ID NO: 26 - DNA, 23 bp, Artificial Sequence
  LPL Reverse
acagagtctgctaatccaggaat